European Patent Application EP 4 715 048 A1, published March 25, 2026. Title: 신규한 PET 분해 효소 및 그 용도. Applicant: 주식회사 자이엔. The sequence listing filed with the application follows.

SEQUENCE LISTING (20 sequences)

SEQ ID NO: 1 - protein, 299 aa, Cryptosporangium aurantiacum
  source 1..299: note = CaPETase WT
MLSFLRSTGRPERRRASLPALLLFTAALVASGLTAAPAAQAADNPYQRGPDPTNASIEAATGPFAVGTQPIVGASGFGGGQIYYPTDTSQTYGAVVIVPGFISVWAQLNWLGPRLASQGFVVIGIETSVITDLPDPRGDQALAALDWATTRSPVASRIDRTRLAAAGWSMGGGGLRRAALQRPSLKAIVGMAPWNGERNWSAVTVPTLFFGGSSDAVASPNDHAKPFYNSITRAEKDYIELRNADHFFPTSANTTMAKYFISWLKRWVDNDTRYTQFLCPGPSTGLFAPVSASMNTCPF

SEQ ID NO: 2 - DNA, 900 bp, Cryptosporangium aurantiacum
  source 1..900: mol_type = genomic DNA; note = CaPETase WT
gtgctgtcctttctccgaagtaccggccgccccgagcgccgacgagcgtcgttaccggcgctcctgttgttcaccgctgcgctcgtcgcgagcgggctcaccgccgcccccgccgcgcaggcggccgacaacccctaccaacgcggtccggaccccacgaacgcgagtatcgaggcggcgaccggcccgttcgcggtcggcacgcagccgatcgtcggtgcctccggcttcggcggcggccagatctactacccgaccgacaccagccagacgtacggggcggtcgtgatcgtgccgggcttcatctcggtctgggcccagctcaactggctcgggccgcgcctggcgtcccagggttttgtggtcatcggcatcgagaccagcgtgatcaccgacctgcccgacccgcgcggtgaccaggcgctggccgcgctggactgggcgacgacccggagcccggtcgcgagccggatcgaccggacccggctggccgcggccggctggtcgatgggcggcggcggcctgcggcgggccgcactgcaacgcccgtcgctcaaggcgatcgtcgggatggcgccctggaacggcgagcgcaactggtccgccgtcaccgtgccgacgctgttcttcggtggttcgtccgacgccgtcgcctcgccgaacgaccacgcgaagccgttctacaacagcatcacccgagccgagaaggattacatcgaactccggaacgccgaccatttcttccccacgtcggcgaacaccacgatggcgaaatacttcatctcgtggctcaagcgttgggtggacaacgacacccgctacacccagttcctctgccccggaccgtccaccggattgttcgccccggtgagcgcgtcgatgaacacctgcccgttctga

SEQ ID NO: 3 - protein, 299 aa, synthetic construct
  source 1..299: note = CaPETaseM1
MLSFLRSTGRPERRRASLPALLLFTAALVASGLTAAPAAQAADNPYQRGPDPTNASIEAATGPFAVGTQPIVGASGFGGGQIYYPTDTSQTYGAVVIVPGFISVWAQLNWLGPRLASQGFVVIGIETSVITDLPDPRGDQALAALDWATTRSPVASRIDRTRLAAAGWSMGGGGLRRAACQRPSLKAIVGMAPWNGERNWSCVTVPTLFFGGSSDAVASPNDHAKPFYNSITRAEKDYIELRNADHFFPTSANTTMAKYFISWLKRWVDNDTRYTQFLCPGPSTGLFAPVSASMNTCPF

SEQ ID NO: 4 - protein, 299 aa, synthetic construct
  source 1..299: note = CaPETaseM2
MLSFLRSTGRPERRRASLPALLLFTAALVASGLTAAPAAQAADNPYQRGPDPTNASIEAATGPFAVGTQPIVGASGFGGGQIYYPTDTSQTYGAVVIVPGFISVWAQLNWLGPRLASQGFVVIGIETSVITDLPDPRGDQALAALDWATTRSPVASRIDRTRLAAAGWSMGGGGLRRAALQRPSLKAIVGMAPWNGERNWSAVTVPTLFFGGSSDAVASPNDHAKPFYNSITRAEKDYIELCNADHFFPTSANTTMAKYFISWLKRWVDNDTRYTQFLCPGPSTGLFAPVCASMNTCPF

SEQ ID NO: 5 - protein, 299 aa, synthetic construct
  source 1..299: note = CaPETaseM3
MLSFLRSTGRPERRRASLPALLLFTAALVASGLTAAPAAQAADNPYQRGPDPTNASIEAATGPFAVGTQPIVGASGFGGGQIYYPTDTSQTYGAVVIVPGFISVWAQLNWLGPRLASQGFVVIGIETSVITDLPDPRGDQALAALDWATTRSPVASRIDRTRLAAAGWSMGGGGLRRAACQRPSLKAIVGMAPWNGERNWSCVTVPTLFFGGSSDAVASPNDHAKPFYNSITRAEKDYIELCNADHFFPTSANTTMAKYFISWLKRWVDNDTRYTQFLCPGPSTGLFAPVCASMNTCPF

SEQ ID NO: 6 - DNA, 33 bp, synthetic construct
  source 1..33: mol_type = other DNA
tatatcatatggcggccgacaacccctaccaac

SEQ ID NO: 7 - DNA, 33 bp, synthetic construct
  source 1..33: mol_type = other DNA
tatatctcgaggaacgggcaggtgttcatcgac

SEQ ID NO: 8 - DNA, 34 bp, synthetic construct
  source 1..34: mol_type = other DNA
tatacatatgcgcggtccgaatccgacagccgcc

SEQ ID NO: 9 - DNA, 34 bp, synthetic construct
  source 1..34: mol_type = other DNA
gcgcctcgaggctgcaattcgctgtacgaaaatc

SEQ ID NO: 10 - DNA, 30 bp, synthetic construct
  source 1..30: mol_type = other DNA
gcgccatatggccaacccctacgaacgtgg

SEQ ID NO: 11 - DNA, 27 bp, synthetic construct
  source 1..27: mol_type = other DNA
gcgcctcgaggaatgggcaggtcgagc

SEQ ID NO: 12 - DNA, 34 bp, synthetic construct
  source 1..34: mol_type = other DNA
tatatcatatgcaatccaacccgtaccagcgcgg

SEQ ID NO: 13 - DNA, 33 bp, synthetic construct
  source 1..33: mol_type = other DNA
tatatctcgagctggcagtggcggttgttcgtc

SEQ ID NO: 14 - protein, 299 aa, synthetic construct
MLSFLRSTGRPERRRASLPALLLFTAALVASGLTAAPAAQAADNPYQRGPDPTNASIEAATGPFAVGTQPIVGASGFGGGQIYYPTDTSQTYGAVVIVPGFISVWAQLAWLGPRLASQGFVVIGIETSVITDLPDPRGDQALAALDWATTRSPVASRIDRTRLAAAGWSMGGGGLRRAACQRPSLKAIVGMAPWNGERNWSCVTVPTLFFGGSSDAVASPNDHAKPFYNSITRAEKDYIELCNADHFFPTSANTTMAKYFISWLKRWVDNDTRYTQFLCPGPSTGLFAPVCASMNTCPF

SEQ ID NO: 15 - protein, 299 aa, synthetic construct
MLSFLRSTGRPERRRASLPALLLFTAALVASGLTAAPAAQAADNPYQRGPDPTNASIEAATGPFAVGTQPIVGASGFGGGQIYYPTDTSQTYGAVVIVPGFISVWAQLNWLGPRLASQGFVVIGIETSVITDLPDPRGDQALAALDWATTRSPVRSRIDRTRLAAAGWSMGGGGLRRAACQRPSLKAIVGMAPWNGERNWSCVTVPTLFFGGSSDAVASPNDHAKPFYNSITRAEKDYIELCNADHFFPTSANTTMAKYFISWLKRWVDNDTRYTQFLCPGPSTGLFAPVCASMNTCPF

SEQ ID NO: 16 - protein, 299 aa, synthetic construct
MLSFLRSTGRPERRRASLPALLLFTAALVASGLTAAPAAQAADNPYQRGPDPTNASIEAATGPFAVGTQPIVGASGFGGGQIYYPTDTSQTYGAVVIVPGFISVWAQLAWLGPRLASQGFVVIGIETSVITDLPDPRGDQALAALDWATTRSPVRSRIDRTRLAAAGWSMGGGGLRRAACQRPSLKAIVGMAPWNGERNWSCVTVPTLFFGGSSDAVASPNDHAKPFYNSITRAEKDYIELCNADHFFPTSANTTMAKYFISWLKRWVDNDTRYTQFLCPGPSTGLFAPVCASMNTCPF

SEQ ID NO: 17 - protein, 299 aa, synthetic construct
MLSFLRSTGRPERRRASLPALLLFTAALVASGLTAAPAAQAADNPYQRGPDPTNASIEAATGPFAVGTQPIVGASGFGGGQIYYPTDTSQTYGAVVIVPGFISVWAQLNWLGPRLASQGFVVIGIETSTITDLPDPRGDQALAALDWATTRSPVASRIDRTRLAAAGWSMGGGGLRRAACQRPSLKAIVGMAPWNGEKNWSCVTVPTLFFGGSSDAVASPNDHAKPFYNSITRAEKDYIELCNADHFFPTSANTTMAKYFISWLKRWVDNDTRYTQFLCPGPSTGLFAPVCASMNTCPF

SEQ ID NO: 18 - protein, 299 aa, synthetic construct
MLSFLRSTGRPERRRASLPALLLFTAALVASGLTAAPAAQAADNPYQRGPDPTNASIEAATGPFAVGTQPIVGASGFGGGQIYYPTDTSQTYGAVVIVPGFISVWAQLNWLGPRLASQGFVVIGIETSTITDLPDPRGDQALAALDWATTRSPVASRIDRTRLAAAGWSMGGGGLRRAACQRPSLKAIVGMAPWNTEKNWSCVTVPTLFFGGSSDAVASPNDHAKPFYNSITRAEKDYIELCNADHFFPTSANTTMAKYFISWLKRWVDNDTRYTQFLCPGPSTGLFAPVCASMNTCPF

SEQ ID NO: 19 - protein, 299 aa, synthetic construct
MLSFLRSTGRPERRRASLPALLLFTAALVASGLTAAPAAQAADNPYQRGPDPTNASIEAATGPFAVGTQPIVGASGFGGGQIYYPTDTSQTYGAVVIVPGFISVWAQLAWLGPRLASQGFVVIGIETSTITDLPDPRGDQALAALDWATTRSPVRSRIDRTRLAAAGWSMGGGGLRRAACQRPSLKAIVGMAPWNGEKNWSCVTVPTLFFGGSSDAVASPNDHAKPFYNSITRAEKDYIELCNADHFFPTSANTTMAKYFISWLKRWVDNDTRYTQFLCPGPSTGLFAPVCASMNTCPF

SEQ ID NO: 20 - protein, 299 aa, synthetic construct
MLSFLRSTGRPERRRASLPALLLFTAALVASGLTAAPAAQAADNPYQRGPDPTNASIEAATGPFAVGTQPIVGASGFGGGQIYYPTDTSQTYGAVVIVPGFISVWAQLAWLGPRLASQGFVVIGIETSTITDLPDPRGDQALAALDWATTRSPVRSRIDRTRLAAAGWSMGGGGLRRAACQRPSLKAIVGMAPWNTEKNWSCVTVPTLFFGGSSDAVASPNDHAKPFYNSITRAEKDYIELCNADHFFPTSANTTMAKYFISWLKRWVDNDTRYTQFLCPGPSTGLFAPVCASMNTCPF